European Patent Application EP 4 722 357 A1, published April 8, 2026. Title: 一种工程化的Cas蛋白及其应用. Applicant: 山东舜丰生物科技有限公司. The sequence listing filed with the application follows.

SEQUENCE LISTING (20 sequences)

SEQ ID NO: 1 - protein, 109 aa, synthetic construct
  REGION 1..109: note = Sa
LIEKIKLHDMQEGKCLYSLEAIPLEDLLNNPFNYEVDHIIPRSVSFDNSFNNKVLVKQEENSKKGNRTPFQYLSSSDSKISYETFKKHILNLAKGKGRISKTKKEYLLE

SEQ ID NO: 2 - protein, 33 aa, synthetic construct
  REGION 1..33: note = Mbps
GKATDVDHIERGDDHSRRNLQAACNRCHGKKSS

SEQ ID NO: 3 - protein, 46 aa, synthetic construct
  REGION 1..46: note = Mbvp
CQSCGHTATPGSGQLHADHIQPRSRGGTDTLDNMRTLCKACHAPKS

SEQ ID NO: 4 - protein, 33 aa, synthetic construct
  REGION 1..33: note = SNF2
NAWHADHIIPVYQGGGECRLENMRTLCVACHAD

SEQ ID NO: 5 - protein, 35 aa, synthetic construct
  REGION 1..35: note = Ps
NAWHADHIIPVYRGGGECNLDNMRTLCVACHSDVT

SEQ ID NO: 6 - protein, 45 aa, synthetic construct
  REGION 1..45: note = Gm
CKRFFNCIGCLCYEYDHIIPFSKGGESTADNCQILQSRVNRLKSD

SEQ ID NO: 7 - protein, 36 aa, synthetic construct
  REGION 1..36: note = Cm
QFWQVDHIKPVYSGGGQCSLENLQTLCTVCHKERTA

SEQ ID NO: 8 - protein, 51 aa, synthetic construct
  REGION 1..51: note = HCTV
CASCGMTRAEHKQVYGRDLHVHHKIPVRVFDDVSDAHFEVNLVTVCMECHE

SEQ ID NO: 9 - protein, 1045 aa, synthetic construct
  REGION 1..1045: note = Cas12i3
MKKVEVSRPYQSLLLPNHRKFKYLDETWNAYKSVKSLLHRFLVCAYGAVPFNKFVEVVEKVDNDQLVLAFAVRLFRLVPVESTSFAKVDKANLAKSLANHLPVGTAIPANVQSYFDSNFDPKKYMWIDCAWEADRLAREMGLSASQFSEYATTMLWEDWLPLNKDDVNGWGSVSGLFGEGKKEDRQQKVKMLNNLLNGIKKNPPKDYTQYLKILLNAFDAKSHKEAVKNYKGDSTGRTASYLSEKSGEITELMLEQLMSNIQRDIGDKQKEISLPKKDVVKKYLESESGVPYDQNLWSQAYRNAASSIKKTDTRNFNSTLEKFKNEVELRGLLSEGDDVEILRSKFFSSEFHKTPDKFVIKPEHIGFNNKYNVVAELYKLKAEATDFESAFATVKDEFEEKGIKHPIKNILEYIWNNEVPVEKWGRVARFNQSEEKLLRIKANPTVECNQGMTFGNSAMVGEVLRSNYVSKKGALVSGEHGGRLIGQNNMIWLEMRLLNKGKWETHHVPTHNMKFFEEVHAYNPSLADSVNVRNRLYRSEDYTQLPSSITDGLKGNPKAKLLKRQHCALNNMTANVLNPKLSFTINKKNDDYTVIIVHSVEVSKPRREVLVGDYLVGMDQNQTASNTYAVMQVVKPKSTDAIPFRNMWVRFVESGSIESRTLNSRGEYVDQLNHDGVDLFEIGDTEWVDSARKFFNKLGVKHKDGTLVDLSTAPRKAYAFNNFYFKTMLNHLRSNEVDLTLLRNEILRVANGRFSPMRLGSLSWTTLKALGSFKSLVLSYFDRLGAKEMVDKEAKDKSLFDLLVAINNKRSNKREERTSRIASSLMTVAQKYKVDNAVVHVVVEGNLSSTDRSASKAHNRNTMDWCSRAVVKKLEDMCNLYGFNIKGVPAFYTSHQDPLVHRADYDDPKPALRCRYSSYSRADFSKWGQNALAAVVRWASNKKSNTCYKVGAVEFLKQHGLFADKKLTVEQFLSKVKDEEILIPRRGGRVFLTTHRLLAESTFVYLNGVKYHSCNADEVAAVNICLNDWVIPCKKKMKEESSASG

SEQ ID NO: 10 - protein, 1228 aa, synthetic construct
  REGION 1..1228: note = Cas12a
MSKLEKFTNCYSLSKTLRFKAIPVGKTQENIDNKRLLVEDEKRAEDYKGVKKLLDRYYLSFINDVLHSIKLKNLNNYISLFRKKTRTEKENKELENLEINLRKEIAKAFKGNEGYKSLFKKDIIETILPEFLDDKDEIALVNSFNGFTTAFTGFFDNRENMFSEEAKSTSIAFRCINENLTRYISNMDIFEKVDAIFDKHEVQEIKEKILNSDYDVEDFFEGEFFNFVLTQEGIDVYNAIIGGFVTESGEKIKGLNEYINLYNQKTKQKLPKFKPLYKQVLSDRESLSFYGEGYTSDEEVLEVFRNTLNKNSEIFSSIKKLEKLFKNFDEYSSAGIFVKNGPAISTISKDIFGEWNVIRDKWNAEYDDIHLKKKAVVTEKYEDDRRKSFKKIGSFSLEQLQEYADADLSVVEKLKEIIIQKVDEIYKVYGSSEKLFDADFVLEKSLKKNDAVVAIMKDLLDSVKSFENYIKAFFGEGKETNRDESFYGDFVLAYDILLKVDHIYDAIRNYVTQKPYSKDKFKLYFQNPQFMGGWDKDKETDYRATILRYGSKYYLAIMDKKYAKCLQKIDKDDVNGNYEKINYKLLPGPNKMLPKVFFSKKWMAYYNPSEDIQKIYKNGTFKKGDMFNLNDCHKLIDFFKDSISRYPKWSNAYDFNFSETEKYKDIAGFYREVEEQGYKVSFESASKKEVDKLVEEGKLYMFQIYNKDFSDKSHGTPNLHTMYFKLLFDENNHGQIRLSGGAELFMRRASLKKEELVVHPANSPIANKNPDNPKKTTTLSYDVYKDKRFSEDQYELHIPIAINKCPKNIFKINTEVRVLLKHDDNPYVIGIDRGERNLLYIVVVDGKGNIVEQYSLNEIINNFNGIRIKTDYHSLLDKKEKERFEARQNWTSIENIKELKAGYISQVVHKICELVEKYDAVIALEDLNSGFKNSRVKVEKQVYQKFEKMLIDKLNYMVDKKSNPCATGGALKGYQITNKFESFKSMSTQNGFIFYIPAWLTSKIDPSTGFVNLLKTKYTSIADSKKFISSFDRIMYVPEEDLFEFALDYKNFSRTDADYIKKWKLYSYGNRIRIFRNPKKNNVFDWEEVCLTSAYKELFNKYGINYQQGDIRALLCEQSDKAFYSSFMALMSLMLQMRNSITGRTDVDFLISPVKNSDGIFYDSRNYEAQENAILPKNADANGAYNIARKVLWAIGQFKKAEDEKLDKVKIAISNKEWLEYAQTSVKH

SEQ ID NO: 11 - protein, 737 aa, synthetic construct
  REGION 1..737: note = Cas-sf0005
MTPKTETPVGALIKKFFPGKRFQKNYLKDAGKKLKREGEAAAVEYLSGKQEDHPANFCPPAKVNILAQSRPLSEWPINLVSKGVQEYVYGLTAAEREANGDFGTSRKSLDRWFARTGVPTHGYTTVQGLNLILRHTFNRYDGVIKKVETRNEKRRSKATRINVSREADGLPPIEAEPEETAFGPDGKLKERPGINPSIYCYQQVSPVPYNPAKHPALPFSGVDPGAPLPLGTPNRLSIPKGQPGYVPEWQRPHLSTKNKRIRKWYARANWRRKPGRKSVLDEAKLKEAALKEAIPIIVTIGKDWIVMDARGLLRAVYWRGIAKPGLSLKELLGFFSGDPVLDPKRGIATFTFKLGAVAVHSRKPTRGKKSKELLLSMTAEKPHVGLVAIDLGQTNPVAAEFSRVKREGETLQAEPLGQIVLPDDLVKDLTRYRRAWDATEEQIKAEAIVQLPEECRAEVVKVNQMSAEETKHLILDRGVSGDLPWEKMTSNTTFISDHLLAKGVTDQVFFEKKSKGKKKGTETVKRKDYGWVKLLRPRLSQETRKAVNDKTWELKRASTEYVRLSRRKTELARRCVNYIVRETKRWTQCEDIAIVIEDLNVRFFHGSGERPDGWDNFFISKRENRWFIQVLHKAFSDLALHRGLPVIEANPARTSITCIRCGHCDRNNRHGEMFLCLSCNDLRHADREIATRNLTRVAVTGEMIPRRIEPGEQSGDTKKARSARKGKKAVISKREAA

SEQ ID NO: 12 - protein, 98 aa, synthetic construct
  REGION 1..98: note = Mbps
MSWSTSDRSSRLPADWEENYRQPVLRAAGYRCQIRQRGCLGKATDVDHIERGDDHSRRNLQAACNRCHGKKSSAEGHARKRQLRARRKRPAERHPGRQ

SEQ ID NO: 13 - protein, 108 aa, synthetic construct
  REGION 1..108: note = Mbvp
MPRAPKVCRHAGCTTLTTTGTCPQHTTHRWGNHQGRKVPHWLQRATFRRDNWTCQSCGHTATPGSGQLHADHIQPRSRGGTDTLDNMRTLCKACHAPKSRAEARGSNT

SEQ ID NO: 14 - protein, 1194 aa, synthetic construct
  REGION 1..1194: note = SNF2
MEVSEEQRRRDEATRLAFAEKRKQSFDSSENPQRQQDFRLAKCRKLDGSNDVCPQEGYRNYEPVRVLSTSVPEKFRVRLEICSPDSFSVTPVQLQGFRCPEEQECLRQLRKILSDAIPLHYTQNDDGGKAGVYKIRDYNKVSGCLKRSKSVEVEGVPWKTLAVVEKLSQSYISGKWQPCLPEHYTEEKVEQLIETLPRKLVNALLPFQLDGLRFGLRRGGRCFIADEMGLGKTLQAIAIAGCFISEGSILVVCPAVLRFTWAEELERWLPSCLPSDVHLVFGHQDNPAYLPRWPKVVVISYKMLQHLRTTMLEREWALLIVDESHHLRCSKKKSDPPEIKTVLDVAEKVKHIILLSGTPSVSRPFDIFHQINMLWPGLLGKDKYEFAKTYCEVGLVRGIQGKIFQDFSKGTRLLELNILLNQTVMIRRLKQHLLTQLPPKRRQIVTILLKKSDIALAMAIVSEAKKQKDGAIAEVTEKSHEPDQNARGSNEAGHVNAENSDGPNSDKENQLCGKLSYQQLGIAKLSAFREWLSLHPLLSGLDYTPEEIDGDRSSTKMVVFAHHHKVLDGIQEFICDKGIGFVRIDGTTLPRDRQLAVQSFQFSSEVKIAIIGVEAGGVGLDFSAAQNVVFLELPKTPSLLLQAEDRAHRRGQTSAVNVYIFCAKDTMDESNWQNLNKKLHRISSTTDGKYDGKTEIEIGGASIFKPAEESSEREVLEGQPSESNTVVADKIVESCDDPGTETDVSNTIDLKDDMTSQLEILEVCPFVENGSGSGMRSSGTISLTMLAQENQENHKPKNLIADDGLVKEVDSSSIFPLIDSLRFEVSQNTGRIHLYSCIPGKDPRPRPHFQNFRPEEIEASNPSQGTTKEKNPESITDDPVHVLAILEFMKEWKSLRPIEKRKLLGKPLQLPLSLELSYLSESTSHNSEGLLRGGSKRRNTPFSEISIPLPENAVWIKVNLRSGHQRKEKEYTQAWSMSNEPLCKLCQKPCAGYNAKEPEYLEDLFCELACYEDYRTRTSSRYIRQELFQIEHGICTNCKLDCHQLVKRLRPLPLEKRRTYINKAAPELFARKNLLETLVNDPTEGNAWHADHIIPVYQGGGECRLENMRTLCVACHADVTAAQCAERKLIRSKARKQLKNTLNELRNNPKQKDLSADENTKETDSATNEEEDELMIEVPGSAYSIDQKINHDAS

SEQ ID NO: 15 - protein, 334 aa, synthetic construct
  REGION 1..334: note = Ps
MMENEAWQNILQAFMKERNGLRPVDQKKLLRKPLQLPLTSELWYLKESINHGSEANDLMPQGLLKGGSKQRNTPLSEISQPLPANASWKKISLCRGRKKEKEYTQGWTVTGEPLCKLCQKPCKGKLSKTPEYFEDLFCEMACFQEYRVKTSQGSLREELFKMEHGVCVACKLDCHELVNYIRPLRYVARGREHVEKVAPNLARSKKLLDKLINYPREGNAWHADHIIPVYRGGGECNLDNMRTLCVACHSDVTKAQSKERRLRNKRGKDRVRDILKGLKLGSSREHNSKEQDDIETRNKEDEDDLLMIDVPGSDYSRATDTVTVSNQENQDEAE

SEQ ID NO: 16 - protein, 162 aa, synthetic construct
  REGION 1..162: note = Gm
MSSSSPQRSRGDGEKRPRFFDSNAKAICWSKADTVPGRHPERWRKDAAGNVVCKRFFNCIGCLCYEYDHIIPFSKGGESTADNCQILQSRVNRLKSDKYNIDSDQLKDYSCEVNFTDKELDIIEMAVYGDVMRPGNQCRCRTIAEKLGKFKPKDDTDACKLP

SEQ ID NO: 17 - protein, 1103 aa, synthetic construct
  REGION 1..1103: note = Cm
MGLGKTIQAIAISYYYKKEWPLLIVVPSSLKYPWIDEMEKWIPELCPDDISIIQNKTDIGRISTSKVTVLGYGLLATDAQTLVDTLYKQNFKIVLVDESHYMKSRNATRSKILLPIVQNAARAILLTGTPALGRPEELFMQIEALFPRRFGTWNEYAKKYCNAHVRFFGKRTLWDCRGASNLDELHQLLSNIMIRRLKNEVLTQLPPKIRQRIPFDLPKAAAKELNTSFEEWEKLMRAPNSDVAESHFVQVMGLITRMYKQTAIAKYTRDKSTSERSPVDSSTPPEREAQAESTGERQLLTYRSEDTRAGAVKDYIKMMLENDKLKFLVFAHHLSMLQACTEAAIENKARYIRIDGSVPSVERIHLVHQFQKDPDTRVAILSIQAAGQGLTFTAATHVVFAELYWDPGHMKQAEDRAHRIGQCSSVNIHYLIAKGTLDPLMWAMLNRKAKVTGSTLNGKKEKLQAEEGDKEKWDFLSFAEAWTPNESLEEVKNEVLFTHFEKEKQHDIRAFFSPKPSAEKKRKIDSWDKSLNFTSGDSKVTPGKDIEEGSRHLDAREIIDVDAICYENGCEPEAKRPRAISTPTQSSSSEKKRKILPGKTNTLFTKESDHGLSGGSLSNSRKKSPLAKVWCCSLCTYTNNSLLPYCEICECPRGSDDKQNTNQMNDPPSTLSEEENASQDSRKIKGIAICNADNERKDLVQTATESSDEIGGEVANAVENGSEECEQKPQEGCVDNSDTFPVYDVLNFCASRNTDRIHLYTKDGKSLNCNFIPLDIKLDNWEDLPESFQQKQNRSLILRFVREWSSLTAMKQKIIRKSGHTFCSPILAAEEISKQQARLSSTKRYVTKEDVAVASLSKANSSGGSVCLVTKEAAFYLKNEGTSAGKTDGHSTKLLLKDGKVSPVLNADSVQAEVVEDPAIYKGYLQAVDNKGNPLCLSCQQPTVHLDQDCKSIAWETRFCSLKCQEDFLIRSSQSYLRSKVFEVEHGVCQLCNLNAQELYLSIKNAPKNQRKNLLESSWMSQLPLGQLNEIITNPAEGQFWQVDHIKPVYSGGGQCSLENLQTLCTVCHKERTAKQAKERSQMKRRSLASKYGSDITKFFVKM

SEQ ID NO: 18 - protein, 248 aa, synthetic construct
  REGION 1..248: note = HCTV
MTKRYQRKDWLEQKYCKESLDKIEIADICGVSRSTVDYWVDKHGVEREYKKSDWLQEKYWEEELSAGEMAEMCEVDRTTILYWMDCHDIERRGFSESSELMWRENEELREEQKERSERVFAESPPPVIADGCHLEETKEKISESLTGKSNPRWRGGSSEYYGGRWDAKREKAILADSEQCASCGMTRAEHKQVYGRDLHVHHKIPVRVFDDVSDAHFEVNLVTVCMECHEEFDRISREWQDRKMEVPA

SEQ ID NO: 19 - protein, 908 aa, synthetic construct
  REGION 1..908: note = Cas12j19
MPSYKSSRVLVRDVPEELVDHYERSHRVAAFFMRLLLAMRREPYSLRMRDGTEREVDLDETDDFLRSAGCEEPDAVSDDLRSFALAVLHQDNPKKRAFLESENCVSILCLEKSASGTRYYKRPGYQLLKKAIEEEWGWDKFEASLLDERTGEVAEKFAALSMEDWRRFFAARDPDDLGRELLKTDTREGMAAALRLRERGVFPVSVPEHLDLDSLKAAMASAAERLKSWLACNQRAVDEKSELRKRFEEALDGVDPEKYALFEKFAAELQQADYNVTKKLVLAVSAKFPATEPSEFKRGVEILKEDGYKPLWEDFRELGFVYLAERKWERRRGGAAVTLCDADDSPIKVRFGLTGRGRKFVLSAAGSRFLITVKLPCGDVGLTAVPSRYFWNPSVGRTTSNSFRIEFTKRTTENRRYVGEVKEIGLVRQRGRYYFFIDYNFDPEEVSDETKVGRAFFRAPLNESRPKPKDKLTVMGIDLGINPAFAFAVCTLGECQDGIRSPVAKMEDVSFDSTGLRGGIGSQKLHREMHNLSDRCFYGARYIRLSKKLRDRGALNDIEARLLEEKYIPGFRIVHIEDADERRRTVGRTVKEIKQEYKRIRHQFYLRYHTSKRDRTELISAEYFRMLFLVKNLRNLLKSWNRYHWTTGDRERRGGNPDELKSYVRYYNNLRMDTLKKLTCAIVRTAKEHGATLVAMENIQRVDRDDEVKRRKENSLLSLWAPGMVLERVEQELKNEGILAWEVDPRHTSQTSCITDEFGYRSLVAKDTFYFEQDRKIHRIDADVNAAINIARRFLTRYRSLTQLWASLLDDGRYLVNVTRQHERAYLELQTGAPAATLNPTAEASYELVGLSPEEEELAQTRIKRKKREPFYRHEGVWLTREKHREQVHELRNQVLALGNAKIPEIRT

SEQ ID NO: 20 - DNA, 2724 bp, synthetic construct
  source 1..2724: mol_type = other DNA
  misc_feature 1..2724: note = Cas12j19
atgcccagctacaagagcagcagagtgctggtgagggacgtgccagaggagctggtggaccactacgaaagaagccacagggtggccgccttcttcatgagactgctgctggccatgagaagagagccctacagcctgagaatgagggacggaaccgagagagaggtggacctggacgaaaccgacgacttcctgagaagcgccggatgcgaggagccagacgccgtgtctgacgacctgagaagcttcgccctggccgtgctgcaccaggacaacccaaagaagagagcctttctggagagcgagaactgcgtgtcaatcctgtgtctggagaaaagcgcctccggcaccagatactacaaaagacccggctaccagctgctgaagaaggccatcgaggaggagtggggatgggacaagttcgaggcctctctgctggacgagagaacaggagaagtggccgagaagttcgccgccctgagcatggaagactggagaagattcttcgccgccagagaccccgacgatctgggaagagagctgctgaagaccgacaccagagaaggcatggccgccgccctgagactgagagaaagaggagtgttccccgtgagcgtgcccgagcacctggacctggacagcctgaaggccgccatggccagcgccgctgaaagactgaagtcatggctggcctgtaaccagcgcgccgtggacgagaagagcgaactgagaaagagattcgaggaggccctggacggagtggaccctgaaaagtatgccctgtttgagaagttcgctgccgagctgcagcaggccgactacaacgtgaccaagaaactggtgctggccgtgagcgccaagttccccgctaccgagcctagcgagtttaagagaggagtggagatcctgaaggaagatggctacaagcccctgtgggaggactttagagagctgggctttgtgtatctggccgagagaaagtgggaaagaagaagaggcggagccgccgtgaccctgtgtgacgctgacgacagccctatcaaggtgagatttggactgactggcagaggcagaaagtttgtgctgtccgccgccgggagcagattcctgatcacagtgaagctgccctgcggcgatgtgggactgaccgccgtgcccagcaggtacttttggaacccctcagtgggcagaaccacctccaactcttttagaattgagttcaccaagcggaccaccgagaatcgcaggtacgtgggcgaggtgaaagagattggcctggtgaggcagagaggcagatactattttttcatcgactacaacttcgacccagaggaggtgagcgacgagaccaaggtgggcagagccttcttcagagcccccctgaacgagtcaagacctaagccaaaggacaagctgaccgtgatggggattgacctgggcattaacccagcctttgcctttgccgtgtgcaccctgggcgaatgccaggacggaatccggagccccgtggccaaaatggaggacgtgagcttcgactctaccggactgagaggcggaatcggcagccagaagctgcacagagagatgcacaacctgagcgacagatgcttttacggcgccagatacattagactgagcaagaagctgagggacagaggagctctgaacgatatcgaggctagactgctggaagagaagtacatccccggctttagaattgtgcacattgaggacgccgacgagagaagaagaaccgtgggaagaacagtgaaagaaatcaaacaggagtacaaaagaatcagacaccagttctacctgaggtaccacaccagcaagagggacagaacagagctgattagcgccgagtacttcagaatgctgttcctggtgaagaacctgagaaacctgctgaagagctggaacagataccactggacaaccggcgacagagaaagaagaggagggaacccagacgagctgaagagctatgtgagatactataacaatctgagaatggacaccctgaagaaactgacctgcgccatcgtgaggaccgccaaggaacacggagccaccctggtggccatggagaacatccagagagtggacagggacgacgaggtgaaaagaagaaaggaaaatagcctgctgagcctgtgggcccccggaatggtgctggagagagtggagcaggagctgaagaacgagggaatcctggcctgggaggtggacccaagacatacaagtcagacaagctgcatcaccgacgaatttggctacagaagcctggtggccaaggacaccttctactttgaacaggacagaaaaatccacagaatcgacgccgacgtgaacgccgccatcaacatcgcccgccgcttcctgacccggtacaggagcctgacccagctgtgggccagcctgctggacgacggcagatacctggtgaacgtgaccagacagcacgagagagcctacctggaactgcagaccggcgcccccgccgctacactgaaccctaccgccgaagccagctacgaactggtgggactgagccccgaagaagaagagctggcccagaccagaatcaaacgcaaaaagagagaaccattctacagacacgaaggcgtgtggctgacaagagagaagcacagagagcaggtgcacgaactgagaaaccaggtgctggccctgggcaacgccaagatccccgaaatcagaacc